European Patent Specification EP 3 656 868 B1, published May 17, 2023. Title: Glucose assay method and glucose sensor. Applicant: Toyobo Co.,Ltd. The sequence listing filed with the application follows.

SEQUENCE LISTING (5 sequences)

SEQ ID NO: 1 - protein, 572 aa, Aspergillus oryzae
MKNTTTYDYIVVGGGTSGLVVANRLSENPDVSVLLLEAGASVFNNPDVTNANGYGLAFGSAIDWQYQSINQSYAGGKQQVLRAGKALGGTSTINGMAYTRAEDVQIDVWQKLGNEGWTWKDLLPYYLKSENLTAPTSSQVAAGAAYNPAVNGKEGPLKVGWSGSLASGNLSVALNRTFQAAGVPWVEDVNGGKMRGFNIYPSTLDVDLNVREDAARAYYFPYDDRKNLHLLENTTANRLFWKNGSAEEAIADGVEITSADGKVTRVHAKKEVIISAGALRSPLILELSGVGNPTILKKNNITPRVDLPTVGENLQDQFNNGMAGEGYGVLAGASTVTYPSISDVFGNETDSIVASLRSQLSDYAAATVKVSNGHMKQEDLERLYQLQFDLIVKDKVPIAEILFHPGGGNAVSSEFWGLLPFARGNIHISSNDPTAPAAINPNYFMFEWDGKSQAGIAKYIRKILRSAPLNKLIAKETKPGLSEIPATAADEKWVEWLKANYRSNFHPVGTAAMMPRSIGGVVDNRLRVYGTSNVRVVDASVLPFQVCGHLVSTLYAVAERASDLIKEDAKSA

SEQ ID NO: 2 - protein, 635 aa, Mucor hiemalis
MKISVAIVTIAAAFASFANAQKTATSNTYDYVIVGGGVGGLALASRLSEDKSVTVAVLEAGPNADEQFVVYAPGMYGQAVGTDLCPLRPTVPQEAMNNRTLTIATGKLLGGGSAINGLVWTRGALKDFDAWEELGNPGWNGRTMFKYFKKVERFHPPTKAQVQYGATYQKGVHGKNGRIDISFPEFQFPQSANWNASLATLDFTHQQDLLNGSLHGYSTTPNTLDPKTARRVDSYTGYIAPFVSRKNLFVLANHTVSRIQFKPKNGTELLKAVGVEWYTTGDNSNKQTIKARREVIVSSGSIGSPKLLEISGIGNKDIVTAAGVQSLIDLPGVGSNMQDHVHAVTVSTTNITGFTTDSVFQNETLAEEQRQQYYNNKTGIWTTTPNNLGYPSPSQLFDGTSFESGQAFANRIRNSTDQWAEYYASTNATNIELLKKQYAIVASRYEENYLSPIEINFTPGYGGTTDVDLKNNKYQTVNHVLIAPLSRGYTHINSSNIEDPVVINPQYYTHPMDVDVHIASTKLARRILGAEPGLASINSGEIQPGSNITSDEDVKQWLADNVRSDWHPVGTCAMLPRELGGVVDPNLLVYGTANLRVVDASIMPLEISSHLMQPTYGVAEKAADIIKMSRKNNNN

SEQ ID NO: 3 - protein, 641 aa, Mucor prainii
MKITAAIITVATAFASFASAQQDTNSSSTDTYDYVTVGGGVAGLALASRISENKDVTVAVLESGPNANDRFVVYAPGMYGQAVGTDLCPLIPTTPQENMGNRSLTIATGRLLGGGSAINGLVWTRGGLKDYDAWEELGNPGWNGANLFKYFKKVENFTPPTPAQIEYGATYQKSAHGKKGPIDVSFTNYEFSQSASWNASLETLDFTALPDILNGTLAGYSTTPNILDPETVQRVDSYTGYIAPYTSRNNLNVLANHTVSRIQFAPKNGSEPLKATGVEWYPTGNKNQKQIIKARYEVIISSGAIGSPKLLEISGIGNKDIVSAAGVESLIDLPGVGSNMQDHVHAITVSTTNITGYTTNSVFVNETLAQEQREEYEANKTGIWATTPNNLGYPTPEQLFNGTEFVSGKEFADKIRNSTDEWANYYASTNASNVELLKKQYAIVASRYEENYLSPIEINFTPGYEGSGNVDLQNNKYQTVNHVLIAPLSRGYTHINSSDVEDHSVINPQYYSHPMDIDVHIASTKLAREIITASPGLGDINSGEIEPGMNITSEDDLRSWLSNNVRSDWHPVGTCAMLPKELGGVVSPALMVYGTSNLRVVDASIMPLEVSSHLMQPTYGIAEKAADIIKNFYKTQHKNQN

SEQ ID NO: 4 - protein, 593 aa, Taralomyces sp.
MLLPSLALAAFSVGAAAKSHHSGSSSSSYHYDYVIVGGGTSGLVVANRLSELHDVTVAVIEAGDSALNNFNVSNVMGYSTAFGTQVDWAYRTENQTYAGGLQQTIRAGKALGGTSTINGMSYTRAEDVQIDIWEVVGNKGWNWTNLLPYYKKSEGFQVPTQDQIAHGANYNASYHGLDGPLKVGWPTSMTNSSVFYALKQTFENLGVDYNPDSAGGKMVGFTDHPDTLDRAKNVREDAARAYYWPYEARSNLKIISNTRANRVVWANSTRGGEAVAVGVEVTNEYGTETIYADREVVLSAGALRSPALLELSGVGNPAVLGQHGIPVRVNLTTVGENLQDQTNNGLSWAGTDTLTGLAAFSALPSVNQLYGDNAADLAASVKSQLASYAQTVAQASKGALREADLLDAFTLQYDLIFKSQVPFTEIVFAPSSQSFAVEYWPLLPFSRGSVHIRSANASDLPAINPNYFMFAQDAEAQVTVAKYIRKALATAPLSGLVDKELSPGLGALPANASSSTWDSWIKANYRTNYHPVGTAIMLPREKGGVVSPELKVYGTKNLRVVDASVLPFQLCGHLTSTLYAVAERASDLIKESH

SEQ ID NO: 5 - protein, 635 aa, Mucor hiemalis NBRC6754; identical to SEQ ID NO: 2